European Patent Specification EP 3 440 051 B1, published March 20, 2024. Title: NEUROPEPTIDE S RECEPTOR (NPSR) AGONISTS. Applicant: RESEARCH TRIANGLE INSTITUTE. The sequence listing filed with the application follows.

SEQUENCE LISTING (1 sequence)

SEQ ID NO: 1 - protein, 20 aa, Human
SFRNGVGTGMKKTSFQRAKS